European Patent Application EP 4 306 635 A1, published January 17, 2024. Title: METHOD FOR OBTAINING INDUCED PLURIPOTENT STEM CELLS (IPSC). Applicant: La Fondation Cardiométabolisme et Nutrition. The sequence listing filed with the application follows.

SEQUENCE LISTING (73 sequences)

SEQ ID NO: 1 - DNA, 20 bp, synthetic construct
  source 1..20: mol_type = other DNA; note = Primer F OCT-4
gtactcctcggtccctttcc

SEQ ID NO: 2 - DNA, 20 bp, synthetic construct
  source 1..20: mol_type = other DNA; note = Primer R OCT-4
caaaaaccctggcacaaact

SEQ ID NO: 3 - DNA, 23 bp, synthetic construct
  source 1..23: mol_type = other DNA; note = Primer F Sox2
ttgctgcctctttaagactagga

SEQ ID NO: 4 - DNA, 20 bp, synthetic construct
  source 1..20: mol_type = other DNA; note = Primer R Sox2
ctggggctcaaacttctctc

SEQ ID NO: 5 - DNA, 22 bp, synthetic construct
  source 1..22: mol_type = other DNA; note = Primer Nanog
ctccaacatcctgaacctcagc

SEQ ID NO: 6 - DNA, 23 bp, synthetic construct
  source 1..23: mol_type = other DNA; note = Primer R Nanog
cgtcacaccattgctattcttcg

SEQ ID NO: 7 - DNA, 23 bp, synthetic construct
  source 1..23: mol_type = other DNA; note = Primer F hTERT
cctgggtggcacggcttttgttc

SEQ ID NO: 8 - DNA, 21 bp, synthetic construct
  source 1..21: mol_type = other DNA; note = Primer R hTERT
cagccttgaagccgcggttga

SEQ ID NO: 9 - DNA, 20 bp, synthetic construct
  source 1..20: mol_type = other DNA; note = Primer F RPL32
agttcctggtccacaacgtc

SEQ ID NO: 10 - DNA, 20 bp, synthetic construct
  source 1..20: mol_type = other DNA; note = Primer R RPL32
gtgactctgatggccagttg

SEQ ID NO: 11 - DNA, 38 bp, synthetic construct
  source 1..38: mol_type = other DNA; note = Primer F Z11p15 H19/IGF2:IG-DMR ICR1
gtttttatattatagtttaagttygttttagttgaggt

SEQ ID NO: 12 - DNA, 28 bp, synthetic construct
  source 1..28: mol_type = other DNA; note = Primer R Z11p15 H19/IGF2:IG-DMR ICR1
tcccataaatattctatccctcactacc

SEQ ID NO: 13 - DNA, 16 bp, synthetic construct
  source 1..16: mol_type = other DNA; note = Probes methylated allele Z11p15 H19/IGF2:IG-DMR ICR1
acgtaacccgaaacgt

SEQ ID NO: 14 - DNA, 20 bp, synthetic construct
  source 1..20: mol_type = other DNA; note = Probes unmethylated allele Z11p15 H19/IGF2:IG-DMR ICR1
cttacataacccaaaacatt

SEQ ID NO: 15 - DNA, 26 bp, synthetic construct
  source 1..26: mol_type = other DNA; note = Primers F 11p15 KCNQ1OT1:TSS-DMR ICR2
gggttagttttttgygtgatgtgttt

SEQ ID NO: 16 - DNA, 20 bp, synthetic construct
  source 1..20: mol_type = other DNA; note = Primer R 11p15 KCNQ1OT1:TSS-DMR ICR2
acctccacaccraaaaccca

SEQ ID NO: 17 - DNA, 21 bp, synthetic construct
  source 1..21: mol_type = other DNA; note = Probe methylated allele 11p15 KCNQ1OT1:TSS-DMR ICR2
atagcggtcgtatttcgatat

SEQ ID NO: 18 - DNA, 20 bp, synthetic construct
  source 1..20: mol_type = other DNA; note = Probes unmethylated allele 11p15 KCNQ1OT1:TSS-DMR ICR2
tgtgtgaggatagtggttgt

SEQ ID NO: 19 - DNA, 33 bp, synthetic construct
  source 1..33: mol_type = other DNA; note = Primer F 14q32 MEG3/DLK1:IG-DMR
agttttatgttaagatgttaattattttttgga

SEQ ID NO: 20 - DNA, 26 bp, synthetic construct
  source 1..26: mol_type = other DNA; note = primer R 14q32 MEG3/DLK1:IG-DMR
accaaaaaacctaacaaatcaaaaca

SEQ ID NO: 21 - DNA, 18 bp, synthetic construct
  source 1..18: mol_type = other DNA; note = Probes methylated allele 14q32 MEG3/DLK1:IG-DMR
tagttcgcggttcgttat

SEQ ID NO: 22 - DNA, 21 bp, synthetic construct
  source 1..21: mol_type = other DNA; note = Probes unmethylated allele 14q32 MEG3/DLK1:IG-DMR
tagtagtttgtggtttgttat

SEQ ID NO: 23 - DNA, 29 bp, synthetic construct
  source 1..29: mol_type = other DNA; note = Primer F 7q32 MEST promoter DMR
gtattagggtgagattagggttattatgg

SEQ ID NO: 24 - DNA, 27 bp, synthetic construct
  source 1..27: mol_type = other DNA; note = Primer R 7q32 MEST promoter DMR
aaatatcactcctacccrcaataaaat

SEQ ID NO: 25 - DNA, 17 bp, synthetic construct
  source 1..17: mol_type = other DNA; note = Probe methylated allele 7q32 MEST promoter DMR
tattacgacgatttcgg

SEQ ID NO: 26 - DNA, 21 bp, synthetic construct
  source 1..21: mol_type = other DNA; note = Probe unmethylated allele 7q32 MEST promoter DMR
aaattttattatgatgatttt

SEQ ID NO: 27 - DNA, 29 bp, synthetic construct
  source 1..29: mol_type = other DNA; note = Primer F 7q12 GRB10:DMR
ggttgtaatatttagttttygagggattg

SEQ ID NO: 28 - DNA, 31 bp, synthetic construct
  source 1..31: mol_type = other DNA; note = Primer R 7q12 GRB10:DMR
crtcacataaatttaatcctaaaattcctat

SEQ ID NO: 29 - DNA, 17 bp, synthetic construct
  source 1..17: mol_type = other DNA; note = Probe methylated allele 7q12 GRB10:DMR
acggagtagcgttcggt

SEQ ID NO: 30 - DNA, 20 bp, synthetic construct
  source 1..20: mol_type = other DNA; note = Probe unmethylated allele 7q12 GRB10:DMR
atggagtagtgtttggtttt

SEQ ID NO: 31 - DNA, 30 bp, synthetic construct
  source 1..30: mol_type = other DNA; note = Primer F 15q11 PWS/AS:DMR
gattttgagyggtgttttatagtttaggtt

SEQ ID NO: 32 - DNA, 24 bp, synthetic construct
  source 1..24: mol_type = other DNA; note = Primer R 15q11 PWS/AS:DMR
tcctataaccttcccacaacrcac

SEQ ID NO: 33 - DNA, 18 bp, synthetic construct
  source 1..18: mol_type = other DNA; note = Probe methylated allele 15q11 PWS/AS:DMR
aacgcatttactacgaac

SEQ ID NO: 34 - DNA, 21 bp, synthetic construct
  source 1..21: mol_type = other DNA; note = Probe unmethylated allele 15q11 PWS/AS:DMR
taacacatttactacaaacca

SEQ ID NO: 35 - DNA, 27 bp, synthetic construct
  source 1..27: mol_type = other DNA; note = Primer F 6q24 PLAGL1:alt-TSS-DMR
aygggttgaatgataaatggtagatgt

SEQ ID NO: 36 - DNA, 18 bp, synthetic construct
  source 1..18: mol_type = other DNA; note = Primer R 6q24 PLAGL1:alt-TSS-DMR
aaccccaacrccctcctc

SEQ ID NO: 37 - DNA, 16 bp, synthetic construct
  source 1..16: mol_type = other DNA; note = Probe methylated allele 6q24 PLAGL1:alt-TSS-DMR
ccgttccgactcccga

SEQ ID NO: 38 - DNA, 19 bp, synthetic construct
  source 1..19: mol_type = other DNA; note = Probe unmethylated allele 6q24 PLAGL1:alt-TSS-DMR
caccattccaactcccaaa

SEQ ID NO: 39 - DNA, 29 bp, synthetic construct
  source 1..29: mol_type = other DNA; note = Primer F 20q13 GNAS/AB:DMR
agtaggggaggttttgtatttttatygta

SEQ ID NO: 40 - DNA, 21 bp, synthetic construct
  source 1..21: mol_type = other DNA; note = Primer R 20q13 GNAS/AB:DMR
tccttacctccaaccacccac

SEQ ID NO: 41 - DNA, 22 bp, synthetic construct
  source 1..22: mol_type = other DNA; note = probe methylated allele 20q13 GNAS/AB:DMR
tcgtaaataattcgaattcggt

SEQ ID NO: 42 - DNA, 18 bp, synthetic construct
  source 1..18: mol_type = other DNA; note = Probe unmethylated allele 20q13 GNAS/AB:DMR
ttggtgggtgtgtgttgt

SEQ ID NO: 43 - DNA, 23 bp, synthetic construct
  source 1..23: mol_type = other DNA; note = Primer F 20q13 GNAS/NESP:DMR
tgtttgggagaggatagaggaga

SEQ ID NO: 44 - DNA, 22 bp, synthetic construct
  source 1..22: mol_type = other DNA; note = Primer R 20q13 GNAS/NESP:DMR
acccccacctccttactacaca

SEQ ID NO: 45 - DNA, 15 bp, synthetic construct
  source 1..15: mol_type = other DNA; note = Probe methylated allele 20q13 GNAS/NESP:DMR
agttgcgcgttcgga

SEQ ID NO: 46 - DNA, 20 bp, synthetic construct
  source 1..20: mol_type = other DNA; note = probe unmethylated allele 20q13 GNAS/NESP:DMR
tgtgaagttgtgtgtttgga

SEQ ID NO: 47 - DNA, 29 bp, synthetic construct
  source 1..29: mol_type = other DNA; note = Primer F 11p15 H19/IGF2:IG-DMR CBS1
ggtttattttgttgattttattaagggag

SEQ ID NO: 48 - DNA, 26 bp, synthetic construct
  source 1..26: mol_type = other DNA; note = Primer R 11p15 H19/IGF2:IG-DMR CBS1
tttctataaataaaccccaaccaaac

SEQ ID NO: 49 - DNA, 23 bp, synthetic construct
  source 1..23: mol_type = other DNA; note = Probes methylated allele 11p15 H19/IGF2:IG-DMR CBS1
atggcgtagaatcggttgtacgt

SEQ ID NO: 50 - DNA, 25 bp, synthetic construct
  source 1..25: mol_type = other DNA; note = Probe unmethylated allele 11p15 H19/IGF2:IG-DMR CBS1
ttagaagtggttgtgtggtggtagt

SEQ ID NO: 51 - DNA, 28 bp, synthetic construct
  source 1..28: mol_type = other DNA; note = Primer F 11p15 H19/IGF2:IG-DMR CBS3
ggatggtatagaatyggttgtaagtgtg

SEQ ID NO: 52 - DNA, 25 bp, synthetic construct
  source 1..25: mol_type = other DNA; note = Primer R 11p15 H19/IGF2:IG-DMR CBS3
aaccccatccaaaaaaaacttaaac

SEQ ID NO: 53 - DNA, 18 bp, synthetic construct
  source 1..18: mol_type = other DNA; note = Probe methylated allele 11p15 H19/IGF2:IG-DMR CBS3
aaaagtggtcgcgcggcg

SEQ ID NO: 54 - DNA, 22 bp, synthetic construct
  source 1..22: mol_type = other DNA; note = Probe unmethylated allele 11p15 H19/IGF2:IG-DMR CBS3
aaagtggttgtgtggtggtagt

SEQ ID NO: 55 - DNA, 27 bp, synthetic construct
  source 1..27: mol_type = other DNA; note = Primer F 11p15 H19/IGF2:IG-DMR CBS4
ggatggtgtagaattggttgtagttgt

SEQ ID NO: 56 - DNA, 28 bp, synthetic construct
  source 1..28: mol_type = other DNA; note = Primer R 11p15 H19/IGF2:IG-DMR CBS4
tcccataaatatcctatccctaataacc

SEQ ID NO: 57 - DNA, 17 bp, synthetic construct
  source 1..17: mol_type = other DNA; note = probe methylated allele 11p15 H19/IGF2:IG-DMR CBS4
tacgaaacccgaaacgt

SEQ ID NO: 58 - DNA, 20 bp, synthetic construct
  source 1..20: mol_type = other DNA; note = Probe unmethylated allele 11p15 H19/IGF2:IG-DMR CBS4
acttacaaaacccaaaacat

SEQ ID NO: 59 - DNA, 25 bp, synthetic construct
  source 1..25: mol_type = other DNA; note = Primer F 11p15 H19/IGF2:IG-DMR CBS5
gtttggatgatttgggatgttttta

SEQ ID NO: 60 - DNA, 25 bp, synthetic construct
  source 1..25: mol_type = other DNA; note = Primer R 11p15 H19/IGF2:IG-DMR CBS5
tctaaaaacttccccttcaatctca

SEQ ID NO: 61 - DNA, 18 bp, synthetic construct
  source 1..18: mol_type = other DNA; note = Probe methylated allele 11p15 H19/IGF2:IG-DMR CBS5
ataactacgcgacgacaa

SEQ ID NO: 62 - DNA, 20 bp, synthetic construct
  source 1..20: mol_type = other DNA; note = Probe unmethylated allele 11p15 H19/IGF2:IG-DMR CBS5
taactacacaacaacaatac

SEQ ID NO: 63 - DNA, 23 bp, synthetic construct
  source 1..23: mol_type = other DNA; note = Primer F 11p15 H19/IGF2:IG-DMR CBS7
tgggttttgggtgttgtttttag

SEQ ID NO: 64 - DNA, 23 bp, synthetic construct
  source 1..23: mol_type = other DNA; note = Primer R 11p15 H19/IGF2:IG-DMR CBS7
caaaacaaacccccacattttac

SEQ ID NO: 65 - DNA, 19 bp, synthetic construct
  source 1..19: mol_type = other DNA; note = Probe methylated allele 11p15 H19/IGF2:IG-DMR CBS7
acggaaatggtcgagaggc

SEQ ID NO: 66 - DNA, 25 bp, synthetic construct
  source 1..25: mol_type = other DNA; note = Probe unmethylated allele 11p15 H19/IGF2:IG-DMR CBS7
agatggaaatggttgagaggtggta

SEQ ID NO: 67 - DNA, 18 bp, synthetic construct
  source 1..18: mol_type = other DNA; note = Primer H19-ex1F
cagtcacccggcccagat

SEQ ID NO: 68 - DNA, 20 bp, synthetic construct
  source 1..20: mol_type = other DNA; note = Primer H19-ex1R
aagacaccatcggaacagca

SEQ ID NO: 69 - DNA, 20 bp, synthetic construct
  source 1..20: mol_type = other DNA; note = primer H19-ex4-5R
gctctggaaggtgaagctag

SEQ ID NO: 70 - DNA, 19 bp, synthetic construct
  source 1..19: mol_type = other DNA; note = Primer H19-ex5-F2
aggccgtctccacaactcc

SEQ ID NO: 71 - DNA, 18 bp, synthetic construct
  source 1..18: mol_type = other DNA; note = Primer DLK1-ex5-F
tgcgtggatgatgagggc

SEQ ID NO: 72 - DNA, 20 bp, synthetic construct
  source 1..20: mol_type = other DNA; note = Primer DLK1-ex5R
cttgcacagacactcgtagc

SEQ ID NO: 73 - DNA, 20 bp, synthetic construct
  source 1..20: mol_type = other DNA; note = Primer DLK1-ex4-5F
tgatcaacggctccccctgc